European Patent Application EP 4 151 597 A1, published March 22, 2023. Title: INORGANIC POROUS SUBSTRATE, INORGANIC POROUS SUPPORT, AND NUCLEIC ACID PRODUCTION METHOD. Applicant: SUMITOMO CHEMICAL COMPANY, LIMITED. Application 21804320.6. The sequence listing filed with the application follows.

SEQUENCE LISTING (1 sequence)

SEQ ID NO: 1 - RNA, 100 nt, Artificial Sequence
  Synthesized RNA
auaacucaauuuguaaaaaaguuuuagagcuagaaauagcaaguuaaaauaaggcuaguccguuaucaacuugaaaaaguggcaccgagucggugcuuuu